European Patent Specification EP 3 982 729 B1, published November 19, 2025. Title: Novel Bacillus thuringiensis strain. Applicant: Bioinsectis S.L. The sequence listing filed with the application follows.

SEQUENCE LISTING (30 sequences)

SEQ ID NO: 1 - DNA, 3456 bp, Bacillus thuringiensis
  CDS (1)..(3456): /note: CDS of cry1Ab24-like gene of B. thuringiensis SVBS-1801, 98% identical to the CDS of gene cry1Ab24 with GenBank accession number HQ439778
  misc_difference (906)..(906): C instead T in the gene cry1Ab24 with GenBank accession number HQ439784
  misc_difference (2379)..(2380): Point where gene cry1Ab24 of accesion number HQ439778 exhibit 78 extra nucleotides
atggataacaatccgaacatcaatgaatgcattccttataattgtttaagtaaccctgaagtagaagtattaggtggagaaagaatagaaactggttacaccccaatcgatatttccttgtcgctaacgcaatttcttttgagtgaatttgttcccggtgctggatttgtgttaggactagttgatataatatggggaatttttggtccctctcaatgggacgcatttcttgtacaaattgaacagttaattaaccaaagaatagaagaattcgctaggaaccaagccatttctagattagaaggactaagcaatctttatcaaatttacgcagaatcttttagagagtgggaagcagatcctactaatccagcattaagagaagagatgcgtattcaattcaatgacatgaacagtgcccttacaaccgctattcctctttttgcagttcaaaattatcaagttcctcttttatcagtatatgttcaagctgcaaatttacatttatcagttttgagagatgtttcagtgtttggacaaaggtggggatttgatgccgcgactatcaatagtcgttataatgatttaactaggcttattggcaactatacagattatgctgtacgctggtacaatacgggattagagcgtgtatggggaccggattctagagattggataagatataatcaatttagaagagaattaacactaactgtattagatatcgtttctctatttccgaactatgatagtagaacgtatccaattcgaacagtttcccaattaacaagagaaatttatacaaacccagtattagaaaattttgatggtagttttcgaggctcggctcagggcatagaaggaagtattaggagtccacatttgatggatatacttagcagtataaccatctatacggatgctcatagaggagaatattattggtcagggcatcaaataatggcttctcctgtagggttttcggggccagaattcacttttccgctatatggaactatgggaaatgcagctccacaacaacgtattgttgctcaactaggtcagggcgtgtatagaacattatcgtccactttatatagaagaccttttaatatagggataaataatcaacaactatctgttcttgacgggacagaatttgcttatgggacctcctcaaatttgccatccgctgtatacagaaaaagcggaacggtagattcgctggatgaaataccaccacagaataacaacgtgccacctaggcaaggatttagtcatcgattaagccatgtttcaatgtttcgttcaggctttagtaatagtagtgtaagtataataagagctcctatgttctcttggatacatcgtagtgctgaatttaataatataattccttcatcacaaattacacaaatacctttaacaaaatctactaatcttggctctggaacttctgtcgttaaaggaccaggatttacaggaggagatattcttcgaagaacttcacctggccagatttcaaccttaagagtaaatattactgcaccattatcacaaagatatcgggtaagaattcgctacgcttctactacaaatttacaattccatacatcaattgacggaagacctattaatcaggggaatttttcagcaactatgagtagtgggagtaatttacagtccggaagctttaggactgtaggttttactactccgtttaacttttcaaatggatcaagtgtatttacgttaagtgctcatgtcttcaattcaggcaatgaagtttatatagatcgaattgaatttgttccggcagaagtaacctttgaggcagaatatgatttagaaagagcacaaaaggcggtgaatgagctgtttacttcttccaatcaaatcgggttaaaaacagatgtgacggattatcatattgatcaagtatccaatttagttgagtgtttatcagatgaattttgtctggatgaaaaacaagaagtgtccgagaaagtcaaacatgcgaagcgacttagtgatgagcggaatttacttcaagatccaaacttcagagggatcaatagacaactagaccgtggctggagaggaagtacggatattaccatccaaggaggcgatgacgtattcaaagagaattacgttacactaccaggtacctttgatgagtgctatccaacgtatttatatcaaaaaatagatgagtcgaaattaaaagcctatacccgttatcaattaagagggtatatcgaggatagtcaagacttagaaatctatttaattcgctacaatgcaaaacatgaaacagtaaatgtgccaggtacgggttccttatggccgctttcagcccaaagtccaatcggaaagtgtgcccatcattcgcatcatttctccttagacattgatgttggatgtacagacttaaatgaggacctaggtgtatgggtgatctttaagattaagacgcaagatgggcacgcaagactagggaatctagagtttctcgaagagaaaccattagtaggagaagcgctagctcgtgtgaaaagagcggagaaaaaatggagagacaaacgcgaaaaattggaatgggaaacaaatatcgtttataaagaggcaaaagaatctgtagatgctttatttgtaaactctcaatatgatcaattacaagcggatacgaatattgccatgattcatgcggcagataaacgtgttcatagcattcgagaagcttatctgcctgagctgtctgtgattccgggtgtcaatgcggctatttttgaagaattagaagggtgtattttcactgcattctccctatatgatgcgagaaatgtcattaaaaatggtgattttaataatggcttatcctgctggaacgtgaaagggcatgtagatgtagaagaacaaaacaaccaccgttcggtccttgttgttccggaatgggaagcagaagtgtcacaagaagttcgtgtctgtccgggtcgtggctatatccttcgtgtcacagcgtacaaggagggatatggagaaggttgcgtaaccattcatgagatcgagaacaatacagacgaactgaagtttagcaactgcgtagaagaggaaatctatccaaacaacacggtaacgtgtaatgattatactgtaaatcaagaagaatacgaaggtgcgtacacttctcgtaatcgaggatataacgaagctccttccgtaccagctgattatgcatcagtctatgaagaaaaatcgtatacagatggacgaagagagaatccttgtgaatttaacagagggtatagggattacacgctactaccagttggttatgtgacaaaagaattagaatacttcccagaaaccgataaggtatggattgagattggagaaacggaaggaacatttatcgtggacagcgtggaattactccttatggaggaataa

SEQ ID NO: 2 - protein, 1151 aa, Bacillus thuringiensis
MDNNPNINECIPYNCLSNPEVEVLGGERIETGYTPIDISLSLTQFLLSEFVPGAGFVLGLVDIIWGIFGPSQWDAFLVQIEQLINQRIEEFARNQAISRLEGLSNLYQIYAESFREWEADPTNPALREEMRIQFNDMNSALTTAIPLFAVQNYQVPLLSVYVQAANLHLSVLRDVSVFGQRWGFDAATINSRYNDLTRLIGNYTDYAVRWYNTGLERVWGPDSRDWIRYNQFRRELTLTVLDIVSLFPNYDSRTYPIRTVSQLTREIYTNPVLENFDGSFRGSAQGIEGSIRSPHLMDILSSITIYTDAHRGEYYWSGHQIMASPVGFSGPEFTFPLYGTMGNAAPQQRIVAQLGQGVYRTLSSTLYRRPFNIGINNQQLSVLDGTEFAYGTSSNLPSAVYRKSGTVDSLDEIPPQNNNVPPRQGFSHRLSHVSMFRSGFSNSSVSIIRAPMFSWIHRSAEFNNIIPSSQITQIPLTKSTNLGSGTSVVKGPGFTGGDILRRTSPGQISTLRVNITAPLSQRYRVRIRYASTTNLQFHTSIDGRPINQGNFSATMSSGSNLQSGSFRTVGFTTPFNFSNGSSVFTLSAHVFNSGNEVYIDRIEFVPAEVTFEAEYDLERAQKAVNELFTSSNQIGLKTDVTDYHIDQVSNLVECLSDEFCLDEKQEVSEKVKHAKRLSDERNLLQDPNFRGINRQLDRGWRGSTDITIQGGDDVFKENYVTLPGTFDECYPTYLYQKIDESKLKAYTRYQLRGYIEDSQDLEIYLIRYNAKHETVNVPGTGSLWPLSAQSPIGKCAHHSHHFSLDIDVGCTDLNEDLGVWVIFKIKTQDGHARLGNLEFLEEKPLVGEALARVKRAEKKWRDKREKLEWETNIVYKEAKESVDALFVNSQYDQLQADTNIAMIHAADKRVHSIREAYLPELSVIPGVNAAIFEELEGCIFTAFSLYDARNVIKNGDFNNGLSCWNVKGHVDVEEQNNHRSVLVVPEWEAEVSQEVRVCPGRGYILRVTAYKEGYGEGCVTIHEIENNTDELKFSNCVEEEIYPNNTVTCNDYTVNQEEYEGAYTSRNRGYNEAPSVPADYASVYEEKSYTDGRRENPCEFNRGYRDYTLLPVGYVTKELEYFPETDKVWIEIGETEGTFIVDSVELLLMEE

SEQ ID NO: 3 - DNA, 3495 bp, Bacillus thuringiensis
  CDS (1)..(3495): /note: CDS of gene of SVBS-1801, 100% identical to CDS of gene cry1Da3 of Genbank accession number: HQ439784
atggaaataaataatcaaaaccaatgtgtgccttacaattgtttaagtaatcctaaggagataatattaggcgaggaaaggctagaaacagggaatactgtagcagacatttcattagggcttattaattttctatattctaattttgtaccaggaggaggatttatagtaggtttactagaattaatatggggatttatagggccttcgcaatgggatatttttttagctcaaattgagcaattgattagtcaaagaatagaagaatttgctaggaatcaggcaatttcaagattggaggggctaagcaatctttataaggtctatgttagagcgtttagcgactgggagaaagatcctactaatcctgctttaagggaagaaatgcgtatacaatttaatgacatgaatagtgctctcataacggctattccactttttagagttcaaaattatgaagttgctcttttatctgtatatgttcaagccgcaaacttacatttatctattttaagggatgtttcagttttcggagaaagatggggatatgatacagcgactatcaataatcgctatagtgatctgactagccttattcatgtttatactaaccattgtgtggatacgtataatcagggattaaggcgtttggaaggtcgttttcttagcgattggattgtatataatcgtttccggagacaattgacaatttcagtattagatattgttgcgttttttccaaattatgatattagaacatatccaattcaaacagctactcagctaacgagggaagtctatctggatttaccttttattaatgaaaatctttctcctgcagcaagctatccaaccttttcagctgctgaaagtgctataattagaagtcctcatttagtagactttttaaatagctttaccatttatacagatagtctggcacgttatgcatattggggagggcacttggtaaattctttccgcacaggaaccactactaatttgataaggtcccctttatatggaagggaaggaaatacagagcgccccgtaactattaccgcatcacctagcgtaccaatatttagaacactttcatatattacaggccttgacaattcaaatcctgtagctggaatcgagggagtggaattccaaaatactataagtagaagtatctatcgtaaaagcggtccaatagattcttttagtgaattaccacctcaagatgccagcgtatctcctgcaattgggtatagtcaccgtttatgccatgcaacatttttagaacggattagtggaccaagaatagcaggcaccgtattttcttggacacaccgtagtgccagccctactaatgaaataagtccatctagaattacacaaattccatgggtaaaggcgcatactcttgcgtctggtgcctccgtcattaaaggtcctggatttacaggtggagatattctgactaggaatagtatgggcgagctggggaccttacgagtaaccttcacaggaagattaccacaaagttattatatacgtttccgttatgcttcggtagcaaataggagtggtacatttagatattcacagccaccttcgtatggaatttcatttccaaaaactatggacgcaggtgaaccactaacatctcgttcgttcgctcatacaacactcttcactccaataaccttttcacgagctcaagaagaatttgatctatacatccaatcgggtgtttatatagatcgaattgaatttattccagttactgcaacatttgaggcagaatatgatttagaaagagcgcaaaaggcggtgaatgccctgtttacgtctacaaaccaactagggctaaaaacaaatgtaacggattatcatattgatcaagtgtccaatttagttgcgtgtttatcggatgaattttgtctggatgaaaagcgagaattgtccgagaaagttaaacatgccaagcgactcagtgatgagcggaatttacttcaagatccaaacttcagaggggtcaataggcaaccagaccgtggctggagaggaagtacggatattaccatccaaggaggagatgatgtattcaaagagaattacgtcacactaccaggtacctttgatgagtgctatccaacgtatttatatcaaaaaatagatgagtcgaagttaaaagcctatacccgttatcaattaagagggtatatcgaggatagtcaagacttagaaatctatttaattcgctacaatgcaaaacacgaaacagtaaacgtgccaggtacaggatccttatggccactttcagccgaaagtccaatcggaaagtgcggagaaccgaatcgatgcgcgccacaccttgaatggaatcctgatttacactgttcctgcagagacggggaaaaatgtgcacatcattctcatcatttctctttggacattgatgttggatgtacagacttacatgatgacttaggtgtatgggtgatattcaagattaagacgcaagatggccacgcacgactagggaatctagagtttctcgaagagaaaccattagtaggagaagcactagctcgtgtgaaaagagcggagaaaaaatggagagacaaacgcgaaacattacaattggaaacaactatcgtttataaagaggcaaaagaatctgtagatgctttatttgtaaactctcaatatgatagattacaagcggatacgaacatcgcgatgattcatgcggcagataaacgcgttcatagaattcgagaagcgtatctgccggagctgtctgtgattccgggtgtcaatgcggctatttttgaagaattagaagggcgtattttcactgcattttccctatatgatgcgagaaatattattaaaaatggcgatttcaataatggcttattgtgctggaacgtgaaagggcatgtagaggtagaagaacaaaacaatcaccgttcagtcctggttatcccagaatgggaggcagaagtgtcacaagaggttcgtgtctgtccaggtcgtggctatatccttcgtgtcacagcgtacaaagagggatatggagagggctgcgtaacgatccatgagatcgaagacaatacagacgaactgaaattcagcaactgtgtagaagaagcatatccaaacaacacggtaacgtgtaatgattatacgacgaaccaagatagatgtgcgggtgtgcacacttctcgtaatcgcggatatgacgaagcctatggaaacaacccttccgtaccagttgattatgcgccagtttataaggaagaagcgtatacagaggtacgaagagataattcttgtgaatctaacagagggtatgggaattatacgccattaccagctggttatgtgacaaaagaattagagtacttcccagaaaccgataaggtatggattgagattggagaaacggaaggaacattcatcgtggatagtgtggaattactcctcatggaggaatag

SEQ ID NO: 4 - protein, 1164 aa, Bacillus thuringiensis
MEINNQNQCVPYNCLSNPKEIILGEERLETGNTVADISLGLINFLYSNFVPGGGFIVGLLELIWGFIGPSQWDIFLAQIEQLISQRIEEFARNQAISRLEGLSNLYKVYVRAFSDWEKDPTNPALREEMRIQFNDMNSALITAIPLFRVQNYEVALLSVYVQAANLHLSILRDVSVFGERWGYDTATINNRYSDLTSLIHVYTNHCVDTYNQGLRRLEGRFLSDWIVYNRFRRQLTISVLDIVAFFPNYDIRTYPIQTATQLTREVYLDLPFINENLSPAASYPTFSAAESAIIRSPHLVDFLNSFTIYTDSLARYAYWGGHLVNSFRTGTTTNLIRSPLYGREGNTERPVTITASPSVPIFRTLSYITGLDNSNPVAGIEGVEFQNTISRSIYRKSGPIDSFSELPPQDASVSPAIGYSHRLCHATFLERISGPRIAGTVFSWTHRSASPTNEISPSRITQIPWVKAHTLASGASVIKGPGFTGGDILTRNSMGELGTLRVTFTGRLPQSYYIRFRYASVANRSGTFRYSQPPSYGISFPKTMDAGEPLTSRSFAHTTLFTPITFSRAQEEFDLYIQSGVYIDRIEFIPVTATFEAEYDLERAQKAVNALFTSTNQLGLKTNVTDYHIDQVSNLVACLSDEFCLDEKRELSEKVKHAKRLSDERNLLQDPNFRGVNRQPDRGWRGSTDITIQGGDDVFKENYVTLPGTFDECYPTYLYQKIDESKLKAYTRYQLRGYIEDSQDLEIYLIRYNAKHETVNVPGTGSLWPLSAESPIGKCGEPNRCAPHLEWNPDLHCSCRDGEKCAHHSHHFSLDIDVGCTDLHDDLGVWVIFKIKTQDGHARLGNLEFLEEKPLVGEALARVKRAEKKWRDKRETLQLETTIVYKEAKESVDALFVNSQYDRLQADTNIAMIHAADKRVHRIREAYLPELSVIPGVNAAIFEELEGRIFTAFSLYDARNIIKNGDFNNGLLCWNVKGHVEVEEQNNHRSVLVIPEWEAEVSQEVRVCPGRGYILRVTAYKEGYGEGCVTIHEIEDNTDELKFSNCVEEAYPNNTVTCNDYTTNQDRCAGVHTSRNRGYDEAYGNNPSVPVDYAPVYKEEAYTEVRRDNSCESNRGYGNYTPLPAGYVTKELEYFPETDKVWIEIGETEGTFIVDSVELLLMEE

SEQ ID NO: 5 - DNA, 3516 bp, Bacillus thuringiensis
  CDS (1)..(3516): /note: CDS of gene of B.thuringiensis SVBS-1801, 100% identical to the CDS of gene cry1Ea7 with GenBank accession number: AY894137
atggagatagtgaataatcagaatcaatgcgtgccttataattgtttaaataatcctgaaaatgagatattagatattgaaaggtcaaatagtactgtagcaacaaacatcgccttggagattagtcgtctgctcgcttccgcaactccaataggggggattttattaggattgtttgatgcaatatgggggtctataggcccttcacaatgggatttatttttagagcaaattgagctattgattgaccaaaaaatagaggaattcgctagaaaccaggcaatttctagattagaagggataagcagtctgtacggaatttatacagaagcttttagagagtgggaagcagatcctactaatccagcattaaaagaagagatgcgtactcaatttaatgacatgaacagtattcttgtaacagctattcctcttttttcagttcaaaattatcaagtcccatttttatcagtatatgttcaagctgcaaatttacatttatcggttttgagagatgtttcagtgtttgggcaggcttggggatttgatatagcaacaataaatagtcgttataatgatctgactagacttattcctatatatacagattatgctgtacgctggtacaatacgggattagatcgcttaccacgaactggtgggctgcgaaactgggcaagatttaatcagtttagaagagagttaacaatatcagtattagatattatttcttttttcagaaattacgattctagattatatccaattccaacaagctcccaattaacgcgggaagtatatacagatccggtaattaatataactgactatagagttggccccagcttcgagaatattgagaactcagccattagaagcccccaccttatggacttcttaaataatttgaccattgatacggatttgattagaggtgttcactattgggcagggcatcgtgtaacttctcattttacaggtagttctcaagtgataacaacccctcaatatgggataaccgcaaatgcggaaccaagacgaactattgctcctagtacttttccaggtcttaacctattttatagaacattatcaaatcctttcttccgaagatcagaaaatattactcctaccttagggataaatgtagtacagggagtagggttcattcaaccaaataatgctgaagttctatatagaagtagggggacagtagattctcttaatgagttaccaattgatggtgagaattcattagttggatatagtcatcgattaagtcatgttacactaaccaggtcgttatataatactaatataactagcctgccaacatttgtttggacacatcacagtgctactaatacaaatacaattaatccagatattattacacaaatacctttagtgaaaggatttagacttggtggtggcacctctgtcattaaaggaccaggatttacaggaggggatatccttcgaagaaataccattggtgagtttgtgtctttacaagtcaatattaactcaccaattacccaaagataccgtttaagatttcgttatgcttccagtagggatgcacgaattactgtagcgataggaggacaaattagagtagatatgacccttgaaaaaaccatggaaattggggagagcttaacatctagaacatttagctataccaattttagtaatcctttttcatttagggctaatccagatataattagaatagctgaagaacttcctattcgtggtggtgagctttatatagataaaattgaacttattctagcagatgcaacatttgaagaagaatatgatttggaaagagcacagaaggcggtgaatgccctgtttacttctacaaatcaactagggctaaaaacagatgtgacggattatcatattgatcaagtttccaatttagttgagtgtttatcggatgaattttgtctggatgaaaagagagaattatccgagaaagtcaaacatgcgaagcgactcagtgatgaacggaatttacttcaagatccaaacttcagagggatcaataggcaaccagaccgtggctggagaggaagcacggatattactatccaaggtggagatgacgtattcaaagagaattacgtcacattaccgggtacctttgatgagtgctatccaacgtatttatatcaaaaaatagatgagtcgaagttaaaagcttatacccgctatgaattaagagggtatatcgaggatagtcaagacttagaaatctatttaattcgctacaatgcaaaacacgagacagtaaacgtgccaggtacgggttccttatggccgctttcagcccaaagtccaatcggaaagtgtggagaaccgaatcgatgcgcgccacaccttgaatggaatcctaatctagattgctcctgcagagacggggaaaaatgtgcccatcattcccatcatttctccttggacattgatgttggatgtacagacttaaatgaggacttaggtgtatgggtgatattcaagattaagacacaagatggctatgcaagactaggaaatctagagtttctcgaagagaaaccactattaggggaagcactagctcgtgtgaaaagagcggagaaaaaatggagagacaaatgcgaaaaattggaatgggaaacaaatattgtttataaagaggcaaaagaatctgtagatgctttatttgtaaactctcaatatgatagattacaagcggatacgaatatcgcgatgattcatgcggcagataaacgcgttcatagcattcgagaagcgtatctgccagagctgtctgtgattccgggtgtcaatgcggctatttttgaagaattagaagggcgtattttcactgcattctccctatatgatgcgagaaatgtcattaaaaatggcgatttcaataatggcttatcatgctggaacgtgaaagggcatgtagatgtagaagaacagaacaaccatcgttcggtccttgttgttccagaatgggaagcagaagtgtcacaagaagttcgtgtttgtccgggtcgtggctatatccttcgtgttacagcgtacaaagagggatatggagagggctgtgtaacgattcatgagatcgaagacaatacagacgaactgaaattcagcaactgtgtagaagaggaagtatatccaaacaacacggtaacgtgtaataattatactgcgactcaagaagaacatgagggtacgtacacttcccgtaatcgaggatatgacgaagcctatgaaagcaattcttctgtacatgcgtcagtctatgaagaaaaatcgtatacagatagacgaagagagaatccttgtgaatctaacagaggatatggggattacacaccactaccagctggctatgtgacaaaagaattagagtacttcccagaaaccgataaggtatggattgagatcggagaaacggaaggaacattcatcgtggacagcgtggaattacttcttatggaggaataa

SEQ ID NO: 6 - protein, 1171 aa, Bacillus thuringiensis
MEIVNNQNQCVPYNCLNNPENEILDIERSNSTVATNIALEISRLLASATPIGGILLGLFDAIWGSIGPSQWDLFLEQIELLIDQKIEEFARNQAISRLEGISSLYGIYTEAFREWEADPTNPALKEEMRTQFNDMNSILVTAIPLFSVQNYQVPFLSVYVQAANLHLSVLRDVSVFGQAWGFDIATINSRYNDLTRLIPIYTDYAVRWYNTGLDRLPRTGGLRNWARFNQFRRELTISVLDIISFFRNYDSRLYPIPTSSQLTREVYTDPVINITDYRVGPSFENIENSAIRSPHLMDFLNNLTIDTDLIRGVHYWAGHRVTSHFTGSSQVITTPQYGITANAEPRRTIAPSTFPGLNLFYRTLSNPFFRRSENITPTLGINVVQGVGFIQPNNAEVLYRSRGTVDSLNELPIDGENSLVGYSHRLSHVTLTRSLYNTNITSLPTFVWTHHSATNTNTINPDIITQIPLVKGFRLGGGTSVIKGPGFTGGDILRRNTIGEFVSLQVNINSPITQRYRLRFRYASSRDARITVAIGGQIRVDMTLEKTMEIGESLTSRTFSYTNFSNPFSFRANPDIIRIAEELPIRGGELYIDKIELILADATFEEEYDLERAQKAVNALFTSTNQLGLKTDVTDYHIDQVSNLVECLSDEFCLDEKRELSEKVKHAKRLSDERNLLQDPNFRGINRQPDRGWRGSTDITIQGGDDVFKENYVTLPGTFDECYPTYLYQKIDESKLKAYTRYELRGYIEDSQDLEIYLIRYNAKHETVNVPGTGSLWPLSAQSPIGKCGEPNRCAPHLEWNPNLDCSCRDGEKCAHHSHHFSLDIDVGCTDLNEDLGVWVIFKIKTQDGYARLGNLEFLEEKPLLGEALARVKRAEKKWRDKCEKLEWETNIVYKEAKESVDALFVNSQYDRLQADTNIAMIHAADKRVHSIREAYLPELSVIPGVNAAIFEELEGRIFTAFSLYDARNVIKNGDFNNGLSCWNVKGHVDVEEQNNHRSVLVVPEWEAEVSQEVRVCPGRGYILRVTAYKEGYGEGCVTIHEIEDNTDELKFSNCVEEEVYPNNTVTCNNYTATQEEHEGTYTSRNRGYDEAYESNSSVHASVYEEKSYTDRRRENPCESNRGYGDYTPLPAGYVTKELEYFPETDKVWIEIGETEGTFIVDSVELLLMEE

SEQ ID NO: 7 - DNA, 3504 bp, Bacillus thuringiensis
  CDS (1)..(3504): /note: CDS of gene cry1Ja1-like of B. thuringiensis SVBS-1801, 94% identical to CDS of gene cry1Ja1 with GenBank accesion number L32019
  misc_difference (987)..(987): T instead of C in gene cry1Ja1 with GenBank accession number L32019, which results in Leu in position 329 of SEQ ID NO:8 replacing Phe in the protein encoded by the CDS of cry1Ja1 gene
  misc_difference (2345)..(2345): G instead of A in gene cry1Ja1 with GenBank accession number L32019, which results in Tyr in position 782 of SEQ ID NO:8 replacing Cys of protein encoded by the CDS of cry1Ja1 gene
atggagataaataatcagaagcaatgcataccatataattgcttaagtaatcctgaggaagtacttttggatggggagaggatattacctgatatcgatccactcgaagtttctttgtcgcttttgcaatttcttttgaataactttgttccagggggaggctttatttcaggattagttgataaaatatggggggctttgagaccatctgaatgggacttatttcttgcacagattgaacggttgattgatcaaagaatagaagcaacagtaagagcaaaagcaatcactgaattagaaggattagggagaaattatcaaatatacgctgaagcatttaaagaatgggaatcagatcctgataacgaagcggctaaaagtagagtaattgatcgctttcgtatacttgatggtctaattgaagcaaatatcccttcatttcggataattggatttgaagtgccacttttatcggtttatgttcaagcagctaatctacatctcgctctattgagagattctgttatttttggagagagatggggattgacgacaaaaaatgtcaatgatatctataatagacaaattagagaaattcatgaatatagcaatcattgcgtagatacgtataacacagaactagaacgtctagggtttagatctatagcgcagtggagaatatataatcagtttagaagagaactaacactaactgtattagatattgtcgctcttttcccgaactatgacagtagactgtatccgatccaaactttttctcaattgacaagagaaattgttacatccccagtaagcgaattttattatggtgttattaatagtggtaatataattggtactcttactgaacagcagataaggcgaccacatcttatggacttctttaactccatgatcatgtatacatcagataatagacgggaacattattggtcaggacttgaaatgacggcttattttacaggacttgcaggagctcaagtgtcattccctttagtcgggactagaggggagtcagctccaccattaactgttagaagtgttaatgatggaatttatagaatattatcggcaccgttttattcagcgccttttctaggcaccattgtattgggaagtcgtggagaaaaatttgattttgcgcttaataatatttcacctccgccatctacaatatacagacatcctggaacagtagattcactagtcagtataccgccacaggataatagcgtaccaccgcacaggggatctagtcatcgattaagtcatgttacaatgcgcgcaagttcccctatattccattggacgcatcgcagcgcaaccactacaaatacaattaatccaaatgctattatccaaataccactagtaaaagcatttaaccttcattcaggtgccactgttgttagaggaccagggtttacaggtggtgatatccttcgaagaacgaatactggcacatttgcagatatgagagtaaatattactgggccattatcccaaagatatcgtgtaagaattcgctatgcttctacgacagatttacaatttttcacgagaatcaatggaacttctgtaaatcaaggtaatttccaaagaactatgaatagaggggataatttagaatctggaaactttaggactgcaggatttagtacgccttttagtttttcaaatgcgcaaagtacattcacattgggtactcaggctttttcaaatcaggaagtttatatagatcgaattgaatttgtcccggcagaagtaacattcgaggcagaatctgatttagaaagagcgcaaaaggcggtgaatgccctgtttacttctacaaaccaactagggctaaaaacagatgtgacggattatcagattgatcaagtgtccaatttagtagaatgtttatcagatgaattttgtctggatgaaaagagagaattgtccgagaaagtcaaacatgcaaagcgacttagtgataagcggaacctacttcaagatccaaacttcacatctatcaatagacaactagaccgtggatggagaggaagtacggatattaccatccaaggaggaaatgacgtattcaaagagaattacgtcacactaccaggtacctttgatgagtgttatccaacgtatttgtatcaaaaaatagatgagtcaaaattaaaagcctatactcgctatgaattaagagggtatattgaagatagtcaagatttagaagtctatttgattcgttacaatgcgaaacatgaaacagtaaatgttcccggtacagggtccttatggccgctttcagtcgaaagcccaatcggaaggtacggagaaccgaatcgatgtgtgccacatattgaatggaatcctgatttagattgttcgtgtagggatggggagaagtgtgcccatcattcgcatcatttctctctagatattgatgttggatgtacagacctaaatgaggacctaggtgtatgggtgatctttaagattaaaacgcaggatggccatgcaagattaggaaatctagagtttctcgaagagaaaccattgttaggagaagcgttagctcgtgtgaaaagagcggagaaaaaatggagagacaaacgcgaacaattgcagtttgaaacgaatatcgtttacaaagaggcaaaagaatctgtagatgctttattcgtagattctcactataatagattacaagcggatacgaacattacgatgattcatgcggcagataaacgcgttcatcgaatccgagaggcttatcttccggaattatccgttatcccaggtgtaaatgcggacatttttgaagaattagaaggtcttattttcactgcattctccctatatgatgcgagaaatatcattaaaaacggtgatttcaataatggtttatcgtgttggaacgtgaaagggcatgtagatatacaacagaatgatcatcgttctgtcctcgttgtcccggaatgggaatcagaggtatcacaagaagtccgcgtatgtccaggtcgtggctatattcttcgtgtcacagcgtacaaagagggctacggagaaggatgcgtaacgatccatgagatcgaagacaatacagacgaattgaagtttagtaactgcatagaagaggaagtctatccaacggatacaggtaatgattatactgcacaccaaggtacaacaggatgcgcagatgcatgtaattcccgtaatgttggatatgaggatggatatgaaataaatactacagcatctgttaattacaaaccgacttatgaagaagaaatgtatacagatgtacgaagagataatcattgtgaatatgacagaggatatgggaaccatacaccgttaccagctggttatgtaacaaaagaattagagtacttccctgaaacagatacagtatggatagagattggagaaacggaaggaacattcatcgtagatagtgtggaattactcctcatggaggaataa

SEQ ID NO: 8 - protein, 1167 aa, Bacillus thuringiensis
MEINNQKQCIPYNCLSNPEEVLLDGERILPDIDPLEVSLSLLQFLLNNFVPGGGFISGLVDKIWGALRPSEWDLFLAQIERLIDQRIEATVRAKAITELEGLGRNYQIYAEAFKEWESDPDNEAAKSRVIDRFRILDGLIEANIPSFRIIGFEVPLLSVYVQAANLHLALLRDSVIFGERWGLTTKNVNDIYNRQIREIHEYSNHCVDTYNTELERLGFRSIAQWRIYNQFRRELTLTVLDIVALFPNYDSRLYPIQTFSQLTREIVTSPVSEFYYGVINSGNIIGTLTEQQIRRPHLMDFFNSMIMYTSDNRREHYWSGLEMTAYFTGLAGAQVSFPLVGTRGESAPPLTVRSVNDGIYRILSAPFYSAPFLGTIVLGSRGEKFDFALNNISPPPSTIYRHPGTVDSLVSIPPQDNSVPPHRGSSHRLSHVTMRASSPIFHWTHRSATTTNTINPNAIIQIPLVKAFNLHSGATVVRGPGFTGGDILRRTNTGTFADMRVNITGPLSQRYRVRIRYASTTDLQFFTRINGTSVNQGNFQRTMNRGDNLESGNFRTAGFSTPFSFSNAQSTFTLGTQAFSNQEVYIDRIEFVPAEVTFEAESDLERAQKAVNALFTSTNQLGLKTDVTDYQIDQVSNLVECLSDEFCLDEKRELSEKVKHAKRLSDKRNLLQDPNFTSINRQLDRGWRGSTDITIQGGNDVFKENYVTLPGTFDECYPTYLYQKIDESKLKAYTRYELRGYIEDSQDLEVYLIRYNAKHETVNVPGTGSLWPLSVESPIGRYGEPNRCVPHIEWNPDLDCSCRDGEKCAHHSHHFSLDIDVGCTDLNEDLGVWVIFKIKTQDGHARLGNLEFLEEKPLLGEALARVKRAEKKWRDKREQLQFETNIVYKEAKESVDALFVDSHYNRLQADTNITMIHAADKRVHRIREAYLPELSVIPGVNADIFEELEGLIFTAFSLYDARNIIKNGDFNNGLSCWNVKGHVDIQQNDHRSVLVVPEWESEVSQEVRVCPGRGYILRVTAYKEGYGEGCVTIHEIEDNTDELKFSNCIEEEVYPTDTGNDYTAHQGTTGCADACNSRNVGYEDGYEINTTASVNYKPTYEEEMYTDVRRDNHCEYDRGYGNHTPLPAGYVTKELEYFPETDTVWIEIGETEGTFIVDSVELLLMEE

SEQ ID NO: 9 - DNA, 2016 bp, Bacillus thuringiensis
  CDS (1)..(2016): /note: CDS of gene of B. thuringiensis SVBS-1801, 100% identical to CDS of gene cry1Nb1 with GenBank accession number KC156678
atgaactcaaatgaacatgattatttgaaagtttgtgatgatttaagtgaaactaatatggagaggtttgacaaaaatgatgcactggagattggtatgtctattgtatctgaacttcttggcatgattccaggcggagcagccttacaatttgtgtttaatcaattgtggtcgcgtttaggtgattctggatggagtgcattcatggaacatgttgaagaattaattgatactaaaatagaagggtatgcaaaaaataaagccttatctgagttagcaggtatgcacagaaatcttgaaacatatataaaattgcttaatgaatgggaaaataatactggaagttcaaaagcacaaggtagagtagctaattattttgaaagtcttgagcaggcggttgaaagaggtatgcctcaattcgcagttggtaatttcgaaataccccttttaactgtttatgtacaagctgctaaccttcatttattgttattaagagatgtttcagtttatggaaaacgctggggatggtcagatcagaaaattaagatttattatgagaaacaagttaagtatactcatgaatacaccaatcattgttcgacttggtataatagaggactagataaattgaaaaataagggttcttcttaccaagattggtacaactataatcgtttccgtagagaaattactcttactgttctagatatcgtcgctgtattcccacactatgatgtgaaagcttatccaattcaaacagttggccaattaacaagggaagtttatacagaccctttaattaattttaatccgcaactagattctgtatctcaattacctacttttagtgatatggaaaatgcaacaattagaaccccacatctgatggagtttttaagaatgctaacaatctatacagattggtatagtgtgggaagaaactattattggggaggacatcgagtgacttcttaccgtgtaggaggagaaaatataacctcccctttatatggaagtgaggcaaatcaagagctgcctagacaactgtatttttatgggccggtttttagaacattatcaaatcctactttaagatacttacagcaacctgcgccagctccgccgtttgctttacgtcgcttagaaggagtagaatttcacaccactacaggtactgatatgtatcgtgaaagaggatcggtagattcttttaatgagctaccgccttttaatccagttggactacctcgtaatgcatatagtcaccgtttatgtcatgcaacgtttgtccgtaaatctgggaccccttatctaataaccggtactgtcttttcttggacacatcgtagtgctgaagaaaccaatacaattgattcaaatagaatcacgcaaattccattggtgaaagcatatcaaattagctcgggcactactgtgaggagaggtccaggattcacaggaggcgatatacttcgaagaactggtcccggtacatttggggatataaaactaaatatcaattcaccattatctcaaagatatcgcgtaaggattcgttatgcttctactactgatttacaatttttcacgaatattaatggaactaccattaatatgggtaatttcccaaaaaccgtgaataattcgagttctgaaggctatagaactgtatcatttagtactccatttagcttttcaaatgcacaaagtatatttagattaggtatacaagctttttctggagtccacgagattcacgttgatagaattgaatttgtcccggcagaggtaacatttgaggcagagtatgatttagaaagggcgcaaaaggcggtaaatgcactatttacatctacaaatccaaaagatatgaaaacatatgtgacagaatctcagattgaccaagtgttcaatctagtagagtgcttatcggacgaggtctgtctcgatgagaagagagaattattcaagaaagtaaaatacgcgaagcaactcaatattgagcgtaacatgtag

SEQ ID NO: 10 - protein, 671 aa, Bacillus thuringiensis
MNSNEHDYLKVCDDLSETNMERFDKNDALEIGMSIVSELLGMIPGGAALQFVFNQLWSRLGDSGWSAFMEHVEELIDTKIEGYAKNKALSELAGMHRNLETYIKLLNEWENNTGSSKAQGRVANYFESLEQAVERGMPQFAVGNFEIPLLTVYVQAANLHLLLLRDVSVYGKRWGWSDQKIKIYYEKQVKYTHEYTNHCSTWYNRGLDKLKNKGSSYQDWYNYNRFRREITLTVLDIVAVFPHYDVKAYPIQTVGQLTREVYTDPLINFNPQLDSVSQLPTFSDMENATIRTPHLMEFLRMLTIYTDWYSVGRNYYWGGHRVTSYRVGGENITSPLYGSEANQELPRQLYFYGPVFRTLSNPTLRYLQQPAPAPPFALRRLEGVEFHTTTGTDMYRERGSVDSFNELPPFNPVGLPRNAYSHRLCHATFVRKSGTPYLITGTVFSWTHRSAEETNTIDSNRITQIPLVKAYQISSGTTVRRGPGFTGGDILRRTGPGTFGDIKLNINSPLSQRYRVRIRYASTTDLQFFTNINGTTINMGNFPKTVNNSSSEGYRTVSFSTPFSFSNAQSIFRLGIQAFSGVHEIHVDRIEFVPAEVTFEAEYDLERAQKAVNALFTSTNPKDMKTYVTESQIDQVFNLVECLSDEVCLDEKRELFKKVKYAKQLNIERNM

SEQ ID NO: 11 - DNA, 1902 bp, Bacillus thuringiensis
  CDS (1)..(1902): /note: CDS of gene of B. thuringiensis SVBS-1801, 100% identical to CDS of gene Cry2Ad1 with Genbank accession number AF200816
atgaatagtgtattgaatagcggaagaaatactatttgtgatgcgtataatgtagtggttcatgatccatttagttttcaacataaatcattagataccatacaaaaagaatggatggagtggaaaaaagataatcatagtttatatgtagatcctattgttggaactgtggctagttttctgttaaagaaattggggagccttattggaaaacggatactgagtgaattacggaatttaatatttcctagtggcagtacaaatctaatggaagatattttaagagagacagaaaaattcctaaatcaaaaacttaatacagacactctttcccgtgtaaatgcggaattgacagggctgcaagcaaatgtagaagagtttaatcgacaagtagataattttttgaaccctaaccgaaacgctgttcctttatcaataacttcttcagttaatacaatgcagcaattatttctaaatagattatcccagttccagatgcaaggataccaactgttattattacctttatttgcacaggcagccaatttacatctttcttttattagagatgttattcttaatgcagaagaatggggcatttcagcagcaacattacgtacgtatcaaaatcacctgagaaattatacaagagattactctaattattgtatagatacgtatcaaactgcgtttagaggtttaaacacccgtttacacgatatgttagaatttagaacatatatgtttttaaatgtatttgaatatgtatctatctggtcgttgtttaaatatcaaagtcttctagtatcttctggcgctaatttatatgcaagtggtagtggaccacagcagacccaattatttacttcacaagactggccatttttatattctcttttccaagttaattcgaattatgtattatccggctttagtggggctagtctttttactacctttcctaatattggtggcttacctggttctactacaactcaagcattacttgctgcaagggttaattatagtggaggaattacatctggtagtatagggggttctaattttaatcaaaattttaattgcaacacgatatcgccacctttgtcaacgtcatttgttagaagttggctagattcgggttcagatcgacagggcgttactaccgttacaaattggcaaacagagtcctttgagacaacttcaggtttaaggtgtggtgcttttacacctcgtggtaattcgaactattaccctggttattttatccgtaatatttctggtgtttctttagttcttagaaatgaagacttaaaaagaccgttatactataacgaaaaaaggaatatagaaagcccttcaggaacacctggtggagcaagagcttatatggtatctgtgcataacaaaaaaaataacatttatgcagttcatgaaaatggtactatgattcatttagcgccggaagataatacaggatttactatatcaccgatacatgccactcaagtgaataatcaaacgcgaacatttatttccgaaaaatttggaaatcaaggtgattccttaagatttgaacaaagcaacacgacagctcgttatacccttagagggaatggaaatagttacaatctttatttaagagtatcttcaataggaaattccactattcgagttactataaacggtagagtttatactgcttcaaatgttaatactactacaaataacgatggagttaatgataacggagctcgtttttcagatattaatatcggtaatgtagtagcaagtagtaattctgatgtaccattagatataaatgtaacattaaactccggtactcaatttgatcttatgaatattatgcttgtaccaactaatatttcaccactttattaa

SEQ ID NO: 12 - protein, 633 aa, Bacillus thuringiensis
MNSVLNSGRNTICDAYNVVVHDPFSFQHKSLDTIQKEWMEWKKDNHSLYVDPIVGTVASFLLKKLGSLIGKRILSELRNLIFPSGSTNLMEDILRETEKFLNQKLNTDTLSRVNAELTGLQANVEEFNRQVDNFLNPNRNAVPLSITSSVNTMQQLFLNRLSQFQMQGYQLLLLPLFAQAANLHLSFIRDVILNAEEWGISAATLRTYQNHLRNYTRDYSNYCIDTYQTAFRGLNTRLHDMLEFRTYMFLNVFEYVSIWSLFKYQSLLVSSGANLYASGSGPQQTQLFTSQDWPFLYSLFQVNSNYVLSGFSGASLFTTFPNIGGLPGSTTTQALLAARVNYSGGITSGSIGGSNFNQNFNCNTISPPLSTSFVRSWLDSGSDRQGVTTVTNWQTESFETTSGLRCGAFTPRGNSNYYPGYFIRNISGVSLVLRNEDLKRPLYYNEKRNIESPSGTPGGARAYMVSVHNKKNNIYAVHENGTMIHLAPEDNTGFTISPIHATQVNNQTRTFISEKFGNQGDSLRFEQSNTTARYTLRGNGNSYNLYLRVSSIGNSTIRVTINGRVYTASNVNTTTNNDGVNDNGARFSDINIGNVVASSNSDVPLDINVTLNSGTQFDLMNIMLVPTNISPLY

SEQ ID NO: 13 - DNA, 2328 bp, Bacillus thuringiensis
  CDS (1)..(2328): /note: CDS of gene of B. thuringiensis SVBS-1801, 100% identical to CDS of gene vip1Ca1 with GenBank accession number AY245547
atgaaaaatatgaagaaaaagttagcaagtgttgtaacgtgtacgttattagctcctatgtttttgaatggaaatgtgaatgctgtttacgcggacagcaaaacaaatcaaatttctacaacacaaaaaaatcaacagaaagagatggaccgaaaaggattacttgggtattatttcaaaggaaaagattttagtaatcttactatgtttgcaccgacacgtgataatactcttatttatgatcaacaaacagcaaataaactattagataaaaaacaacaacaatatcagtctattcgttggattggtttgattcagagtaaagaaaagggagatttcacatttaacttatctgaggatgaacaggcaattatagaaatcgatggaaaaatcatttctaataaagggaaagaaaagcaagttgtccatttagaaaaagaaaaattagttccaatcaaaatagagtatcaatcagatacgaaatttaatattgacagtaaaacatttaaagaatttaaattatttaaaatagatagtcaaaaccaatcccaacaagtcaaacgagatgaactcagaaaccctgaatttaacaaaaaagaatcacgggaattcttagcaaaagcatcaaaaacaaatttttttatgcaaaaaatgaaaagagatattgatgaagatacggatacagatggcgactccattcctgatctttgggaagaaaacgggtacacgattcaaaataaggtcgctgtaaaatgggatgataaatttgctcaacaagggtatgttaaatatttatcaagcccttatcaagctcatacagttggagatccttacactgactgggaaaaagcagctggagatattccaaaatctaatgcagctgcaacacgtaatccattagtagcagcttttcctagtataaatgtcgatatgaggaaaatgattttatctaaggattctaatttatcgaattccgctgaggcccattcaaataatagctatacttatgcaaatagtgaaggggcaagtattgaagctggctttggtcctaaaggattttcttttggggtcagtgctaattatcaacatacagaaacagttggttctgattggggaaattctaaaagtaacacagagcaatttaattctgcttcagctggttacttaaatgctaatgtccattataataatgtgggaactggtggaatatatgatgctcaaccaaccactagttttattttgcaagactctacaattgctaccattacagcaaaatctaatgctactgctttaagcataccatcaggagatcgataccctgcgagcaaagaaggaatttctttaaaaactatggatgattttaattcccatcctattactttaaacaaaccacaattagatgcagtattaaacaatgaggtaataaagataaatactgatcaaactgatggtagatatggaataattggagtggatggtaaggctgaaataggtgatcgatggagtccgattatagacgaaataaagggaagaacagcttcaattattattgatcctgctgacggaaaagctttagaaacaagaatagctgctaaagattataaaaatcctgaagataaaactccaagtttaacaattaaagaaggacttaaaatagcatatcctgaatcgattagtgaagataaagatggaatactattttatgaatataaaaatgatgaaggtaaagtcactaaaaaacaacttagtgaagagaatattatgccttatttagatgaagatacttcaaaagaattcgagagacaattatctgatgggagtgctaaaggattatatgatataaaactaacacctaaaatgaatattactatcagattagctactgtgacacttggatttgatgatcaatttagtgcttatccatgggaaaatgcaacttggtctgataaattcgggaatcttagacttggttctttagctatacctcaagagtctaaatataccattcctaaagataaagtaaaaccaaattatgattatttaattactggttatataaaacatgattttacaacagataatgaatcattaggtatagtcgccttcacgaaaaaggataattttgaaatgtggaacatggggacatcaattttttcacaaaattctggaggtgaatttaaaaaattcactataaaaacacaaaatatttctggagattatatacttgattccattcaattaatgaagagaaataatgatgtaaataagatagatagctatcttgatgatatttcaattatccctataggacctaacaaatctagataa

SEQ ID NO: 14 - protein, 775 aa, Bacillus thuringiensis
MKNMKKKLASVVTCTLLAPMFLNGNVNAVYADSKTNQISTTQKNQQKEMDRKGLLGYYFKGKDFSNLTMFAPTRDNTLIYDQQTANKLLDKKQQQYQSIRWIGLIQSKEKGDFTFNLSEDEQAIIEIDGKIISNKGKEKQVVHLEKEKLVPIKIEYQSDTKFNIDSKTFKEFKLFKIDSQNQSQQVKRDELRNPEFNKKESREFLAKASKTNFFMQKMKRDIDEDTDTDGDSIPDLWEENGYTIQNKVAVKWDDKFAQQGYVKYLSSPYQAHTVGDPYTDWEKAAGDIPKSNAAATRNPLVAAFPSINVDMRKMILSKDSNLSNSAEAHSNNSYTYANSEGASIEAGFGPKGFSFGVSANYQHTETVGSDWGNSKSNTEQFNSASAGYLNANVHYNNVGTGGIYDAQPTTSFILQDSTIATITAKSNATALSIPSGDRYPASKEGISLKTMDDFNSHPITLNKPQLDAVLNNEVIKINTDQTDGRYGIIGVDGKAEIGDRWSPIIDEIKGRTASIIIDPADGKALETRIAAKDYKNPEDKTPSLTIKEGLKIAYPESISEDKDGILFYEYKNDEGKVTKKQLSEENIMPYLDEDTSKEFERQLSDGSAKGLYDIKLTPKMNITIRLATVTLGFDDQFSAYPWENATWSDKFGNLRLGSLAIPQESKYTIPKDKVKPNYDYLITGYIKHDFTTDNESLGIVAFTKKDNFEMWNMGTSIFSQNSGGEFKKFTIKTQNISGDYILDSIQLMKRNNDVNKIDSYLDDISIIPIGPNKSR

SEQ ID NO: 15 - DNA, 1389 bp, Bacillus thuringiensis
  CDS (1)..(1389): /note: CDS of gene of B. thuringiensis SVBS-1801, 100% identical to CDS of gene vip2Ac1 with GenBank accession number AY245547
atgaaaagaatggagggaaaattgtttatggtgtccacaaaattacaagcagttactaaagctgtattacttagtacagttttatctatatctttattaaataatgaagtgataaaagctgaacaattaaatatgaattctcaaaataaatatactaattttgaaaatctaaaaatcactgacaaggtagaggattttaaagaagataaggaaaaagcgaaagaatgggggaaagaaaaagaaaaagagtggaaactaactgctactgaaaaaggaaaaatgaataattttttagataataaaaatgatataaaaacaaattataaagaaattactttttctatggcaggttcatttgaagatgaaataaaagatttaaaagaaattgataagatctttgataaagccaatctctcaagtcctattatcacctataaaaatgtggaaccagcaacaattggatttaataaatctttaacagaaggtaatacaattaattctgatgcaatggcacagtttaaagaacaatttttagatagggatattaagtttgatagttatctggatacgcatttaactgttcaacaagtttccagtaaagaaagagttattttgaaggttaaggttccgagtggaaaaggttctactactccaacaaaagcaggtatcattttaaataatagtgaatacaaaatgcttattgataatgggtatatggtccatgtagataaggtgtcaaaagtggtaaaaaaaggggtggagtgcttacaagttgaagggactttaaaaaagagtcttgattttaaaaatgatataaatgctggagcgcatagctggggtatgaagaattatgaagagtgggctaaagatttaaccgatttacaaagggaagctttagatgggtatgctaggcaagattataaagaaatcaataattatttacgaaatcaaggcggaaatggaaatgaaaaactagatgctcaaataaaaaatatttctgatgctttagggaagaaaccaataccggaaaatattactgtgtatagatggtgtggcatgccggaatttggttatcaaattagtgatccgttaccttctttaaaagattttgaagaacaatttttaaatacaatcaaagaagacaaaggatatatgagtacaagcttatcgagtgaacgtcttgcagcttttggatctagaaaaattatattacgattacaagttccgaaaggaagtacgggtgcgtatttaagtgccataggtggatttgcaaatgaaaaagagatactacttgataaagatagtaaatatcatattgataaagtaacagaggtaattattaaaggtgttaagcgatatgtagtggatgcaacattattaacaaattaa

SEQ ID NO: 16 - protein, 462 aa, Bacillus thuringiensis
MKRMEGKLFMVSTKLQAVTKAVLLSTVLSISLLNNEVIKAEQLNMNSQNKYTNFENLKITDKVEDFKEDKEKAKEWGKEKEKEWKLTATEKGKMNNFLDNKNDIKTNYKEITFSMAGSFEDEIKDLKEIDKIFDKANLSSPIITYKNVEPATIGFNKSLTEGNTINSDAMAQFKEQFLDRDIKFDSYLDTHLTVQQVSSKERVILKVKVPSGKGSTTPTKAGIILNNSEYKMLIDNGYMVHVDKVSKVVKKGVECLQVEGTLKKSLDFKNDINAGAHSWGMKNYEEWAKDLTDLQREALDGYARQDYKEINNYLRNQGGNGNEKLDAQIKNISDALGKKPIPENITVYRWCGMPEFGYQISDPLPSLKDFEEQFLNTIKEDKGYMSTSLSSERLAAFGSRKIILRLQVPKGSTGAYLSAIGGFANEKEILLDKDSKYHIDKVTEVIIKGVKRYVVDATLLTN

SEQ ID NO: 17 - DNA, 2367 bp, Bacillus thuringiensis
  CDS (1)..(2367): /note: CDS of gene of B. thuringiensis SVBS-1801, 100% identical to CDS of gene vip3Af3 with GenBank accession number HM117634
atgaatatgaataatactaaattaaacgcaagggccctaccgagttttattgattattttaatggcatttatggatttgccactggtatcaaagacattatgaatatgatttttaaaacggatacaggtggtaatctaaccttagacgaaatcctaaagaatcagcagttactaaatgagatttctggtaaattggatggggtaaatgggagcttaaatgatcttatcgcacagggaaacttaaatacagaattatctaaggaaatcttaaaaattgcaaatgaacagaatcaagtcttaaatgatgttaataacaaactcgatgcgataaatacgatgcttcatatatatctacctaaaattacatctatgttaagtgatgtaatgaagcaaaattatgcgctaagtctgcaaatagaatacttaagtaagcaattgcaagaaatttctgataaattagatattattaacgtaaatgttcttattaactctacacttactgaaattacacctgcatatcaacggattaaatatgtgaatgaaaaatttgaagaattaacttttgctacagaaaccactttaaaagtaaaaaaggatagctcgcctgctgatattcttgatgagttaactgaattaactgaactagcgaaaagtgttacaaaaaatgacgttgatggttttgaattttaccttaatacattccacgatgtaatggtaggaaataatttattcgggcgttcagctttaaaaactgcttcagaattaattgctaaagaaaatgtgaaaacaagtggcagtgaagtaggaaatgtttataatttcttaattgtattaacagctctacaagcaaaagcttttcttactttaacaacatgccgaaaattattaggcttagcagatattgattatacttctattatgaatgaacatttaaataaggaaaaagaggaatttagagtaaacatccttcctacactttctaatactttttctaatcctaattatgcaaaagttaaaggaagtgatgaagatgcaaagatgattgtggaagctaaaccaggacatgcattggttgggtttgaaatgagcaatgattcaatcacagtattaaaagtatatgaggctaagctaaaacaaaattatcaagttgataaggattccttatcggaggttatttatggtgatacggataaattattttgtccagatcaatctgaacaaatatattatacaaataacatagtattcccaaatgaatatgtaattactaaaattgatttcactaaaaaaatgaaaactttaagatatgaggtaacagcgaatttttatgattcttctacaggagaaattgacttaaataagaaaaaagtagaatcaagtgaagcggagtatagaacgttaagtgctaatgatgatggagtgtatatgccattaggtgtcatcagtgaaacatttttgactccgataaatgggtttggcctccaagctgatgaaaattcaagattaattactttaacatgtaaatcatatttaagagaactactgctagcaacagacttaagcaataaagaaactaaattgatcgtcccaccaagtggttttattagcaatattgtagagaacgggtccatagaagaggacaatttagagccgtggaaagcaaataataagaatgcgtatgtagatcatacaggcggagtgaatggaactaaagctttatatgttcataaggacggaggattttcacaatttattggagataagttaaaaccgaaaactgagtatgtaatccaatatactgttaaaggaaaaccttctattcatttaaaagatgaaaatactggatatattcattatgaagatacaaataataatttaaaagattatcaaactattactaaacgttttactacaggaactgatttaaagggagtgtatttaattttaaaaagtcaaaatggagatgaagcttggggagataaatttacaattttagaaattaagcctgcggaggatttattaagcccagaattaattaatccgaattcttggattacgactccaggggctagcatttcaggaaataaacttttcattaacttggggacaaatgggacctttagacaaagtctttcattaaacagttattcaacttatagtataagctttactgcatcaggaccatttaatgtgacggtaagaaattctagggaagtattatttgaacgaagcaaccttatgtcttcaactagtcatatttctgggacattcaaaactgaatccaataataccggattatatgtagaactttcccgtcgctctggtggtggtggtcatatatcatttgaaaacgtttctattaaataa

SEQ ID NO: 18 - protein, 788 aa, Bacillus thuringiensis
MNMNNTKLNARALPSFIDYFNGIYGFATGIKDIMNMIFKTDTGGNLTLDEILKNQQLLNEISGKLDGVNGSLNDLIAQGNLNTELSKEILKIANEQNQVLNDVNNKLDAINTMLHIYLPKITSMLSDVMKQNYALSLQIEYLSKQLQEISDKLDIINVNVLINSTLTEITPAYQRIKYVNEKFEELTFATETTLKVKKDSSPADILDELTELTELAKSVTKNDVDGFEFYLNTFHDVMVGNNLFGRSALKTASELIAKENVKTSGSEVGNVYNFLIVLTALQAKAFLTLTTCRKLLGLADIDYTSIMNEHLNKEKEEFRVNILPTLSNTFSNPNYAKVKGSDEDAKMIVEAKPGHALVGFEMSNDSITVLKVYEAKLKQNYQVDKDSLSEVIYGDTDKLFCPDQSEQIYYTNNIVFPNEYVITKIDFTKKMKTLRYEVTANFYDSSTGEIDLNKKKVESSEAEYRTLSANDDGVYMPLGVISETFLTPINGFGLQADENSRLITLTCKSYLRELLLATDLSNKETKLIVPPSGFISNIVENGSIEEDNLEPWKANNKNAYVDHTGGVNGTKALYVHKDGGFSQFIGDKLKPKTEYVIQYTVKGKPSIHLKDENTGYIHYEDTNNNLKDYQTITKRFTTGTDLKGVYLILKSQNGDEAWGDKFTILEIKPAEDLLSPELINPNSWITTPGASISGNKLFINLGTNGTFRQSLSLNSYSTYSISFTASGPFNVTVRNSREVLFERSNLMSSTSHISGTFKTESNNTGLYVELSRRSGGGGHISFENVSIK

SEQ ID NO: 19 - DNA, 31 bp, Artificial sequence
  Primer Fwd-SaI for amplification of cry1Ab24-like gen
ggtcgacggtatcttaataaaagagatggag

SEQ ID NO: 20 - DNA, 33 bp, Artificial sequence
  Primer Rev-PaeI for amplification of cry1Ab24-like gene
gcatgcttattcctccataaggagtaattccac

SEQ ID NO: 21 - DNA, 35 bp, Artificial sequence
  Forward primer for amplification of gene cry1Da3
ggtcgacggactttagtaatttaataaaaaaaggg

SEQ ID NO: 22 - DNA, 33 bp, Artificial sequence; identical to SEQ ID NO: 20
  Reverse primer for amplification of gene cry1Da3

SEQ ID NO: 23 - DNA, 33 bp, Artificial sequence
  Forward primer for amplification of gene cry1Ea7
gtgtcgaccagtaccaaattataagaactttgg

SEQ ID NO: 24 - DNA, 33 bp, Artificial sequence; identical to SEQ ID NO: 20
  Reverse primer for amplification of gene cry1Ea7

SEQ ID NO: 25 - DNA, 28 bp, Artificial sequence
  Forward primer for amplification of gene cry1Ja1-like
ggtcgacaaccaaagagaaaggggtaac

SEQ ID NO: 26 - DNA, 29 bp, Artificial sequence
  Reverse primer for amplification of gene cry1Ja1-like
ggcatgcgttacagagattagacgactac

SEQ ID NO: 27 - DNA, 33 bp, Artificial sequence
  Forward primer for amplification of gene cry1Nb1
gtcgacctaaaaataatgaatattggaggaaag

SEQ ID NO: 28 - DNA, 30 bp, Artificial sequence
  Reverse primer for amplification of gene cry1Nb1
ctgcagctacatgttacgctcaatattgag

SEQ ID NO: 29 - DNA, 36 bp, Artificial sequence
  Forward primer for amplification of gene cry2Ad1
gtgtcgaccctaatatttaaggaggaattttatatg

SEQ ID NO: 30 - DNA, 30 bp, Artificial sequence
  Reverse primer for amplification of gene cry2Ad1
gcgcatgcctcaaactttaataaagtggtg